European Patent Application EP 4 163 294 A1, published April 12, 2023. Title: Modified ferritin and production method thereof. Applicant: Ajinomoto Co., Inc. The sequence listing filed with the application follows.

SEQUENCE LISTING (20 sequences)

SEQ ID NO: 1 - protein, 183 aa, Homo sapiens
MTTASTSQVRQNYHQDSEAAINRQINLELYASYVYLSMSYYFDRDDVALKNFAKYFLHQSHEEREHAEKLMKLQNQRGGRIFLQDIKKPDCDDWESGLNAMECALHLEKNVNQSLLELHKLATDKNDPHLCDFIETHYLNEQVKAIKELGDHVTNLRKMGAPESGLAEYLFDKHTLGDSDNES

SEQ ID NO: 2 - DNA, 552 bp, Homo sapiens
atgacgaccgcgtccacctcgcaggtgcgccagaactaccaccaggactcagaggccgccatcaaccgccagatcaacctggagctctacgcctcctacgtttacctgtccatgtcttactactttgaccgcgatgatgtggctttgaagaactttgccaaatactttcttcaccaatctcatgaggagagggaacatgctgagaaactgatgaagctgcagaaccaacgaggtggccgaatcttccttcaggatatcaagaaaccagactgtgatgactgggagagcgggctgaatgcaatggagtgtgcattacatttggaaaaaaatgtgaatcagtcactactggaactgcacaaactggccactgacaaaaatgacccccatttgtgtgacttcattgagacacattacctgaatgagcaggtgaaagccatcaaagaattgggtgaccacgtgaccaacttgcgcaagatgggagcgcccgaatctggcttggcggaatatctctttgacaagcacaccctgggagacagtgataatgaaagctaa

SEQ ID NO: 3 - protein, 182 aa, Homo sapiens
TTASTSQVRQNYHQDSEAAINRQINLELYASYVYLSMSYYFDRDDVALKNFAKYFLHQSHEEREHAEKLMKLQNQRGGRIFLQDIKKPDCDDWESGLNAMECALHLEKNVNQSLLELHKLATDKNDPHLCDFIETHYLNEQVKAIKELGDHVTNLRKMGAPESGLAEYLFDKHTLGDSDNES

SEQ ID NO: 4 - DNA, 36 bp, Artificial Sequence
  Primer
gaaggagatatacatatgacgaccgcgtccacctcg

SEQ ID NO: 5 - DNA, 36 bp, Artificial Sequence
  Primer
ctcgaattcggatccttagctttcattatcactgtc

SEQ ID NO: 6 - DNA, 33 bp, Artificial Sequence
  Primer
tttcatatgtatatctccttcttaaagttaaac

SEQ ID NO: 7 - DNA, 26 bp, Artificial Sequence
  Primer
tttggatccgaattcgagctccgtcg

SEQ ID NO: 8 - protein, 29 aa, Artificial Sequence
  Peptide fragment of human ferritin H chain
IFLQDIKKPDCDDWESGLNAMECALHLEK

SEQ ID NO: 9 - protein, 22 aa, Artificial Sequence
  Peptide fragment of human ferritin H chain
KPDCDDWESGLNAMECALHLEK

SEQ ID NO: 10 - protein, 11 aa, Artificial Sequence
  One example of peptide to be encapsulated in human ferritin
CGGPKKKRKVG

SEQ ID NO: 11 - DNA, 18 bp, Artificial Sequence
  One example of DNA to be encapsulated in human ferritin
aacaggtaggttcagtgt

SEQ ID NO: 12 - DNA, 18 bp, Artificial Sequence
  One example of DNA to be encapsulated in human ferritin
acactgaacctacctgtt

SEQ ID NO: 13 - protein, 11 aa, Artificial Sequence
  One example of peptide to be encapsulated in human ferritin
YGRKKRRQRRR

SEQ ID NO: 14 - protein, 9 aa, Artificial Sequence
  One example of peptide to be encapsulated in human ferritin
RRRRRRRRR

SEQ ID NO: 15 - RNA, 19 nt, Artificial Sequence
  Sense strand of siRNA
acagcaaauuccaucgugu

SEQ ID NO: 16 - RNA, 21 nt, Artificial Sequence
  Antisense strand of siRNA
acacgauggaauuugcuguuu

SEQ ID NO: 17 - protein, 16 aa, Artificial Sequence
  Gold-binding peptide 1 (GBP1)
GMHGKTQATSGTIQSG

SEQ ID NO: 18 - DNA, 576 bp, Artificial Sequence
  Polynucleotide encoding fusion protein of human ferritin H chain and gold-binding peptide inserted into a flexible linker portion between 2nd and 3rd alpha-helices of human ferritin H chain from N-terminus
atgacgaccgcgtccacctcgcaggtgcgccagaactaccaccaggactcagaggccgccatcaaccgccagatcaacctggagctctacgcctcctacgtttacctgtccatgtcttactactttgaccgcgatgatgtggctttgaagaactttgccaaatactttcttcaccaatctcatgaggagagggaacatgctgagaaactgatgaagctgcagaaccaacgaggtggccgaatcttccttcaggatatcaagggtcgcaaacttccggatgcgggcaaaccagactgtgatgactgggagagcgggctgaatgcaatggagtgtgcattacatttggaaaaaaatgtgaatcagtcactactggaactgcacaaactggccactgacaaaaatgacccccatttgtgtgacttcattgagacacattacctgaatgagcaggtgaaagccatcaaagaattgggtgaccacgtgaccaacttgcgcaagatgggagcgcccgaatctggcttggcggaatatctctttgacaagcacaccctgggagacagtgataatgaaagctaa

SEQ ID NO: 19 - protein, 199 aa, Artificial Sequence
  Fusion protein of human ferritin H chain and gold-binding peptide inserted into a flexible linker portion between 2nd and 3rd alpha-helices of human ferritin H chain from N-terminus
MTTASTSQVRQNYHQDSEAAINRQINLELYASYVYLSMSYYFDRDDVALKNFAKYFLHQSHEEREHAEKLMKLQNQRGGRIFLQDIKGMHGKTQATSGTIQSGKPDCDDWESGLNAMECALHLEKNVNQSLLELHKLATDKNDPHLCDFIETHYLNEQVKAIKELGDHVTNLRKMGAPESGLAEYLFDKHTLGDSDNES

SEQ ID NO: 20 - protein, 198 aa, Artificial Sequence
  Fusion protein of human ferritin H chain and gold-binding peptide inserted into a flexible linker portion between 2nd and 3rd alpha-helices of human ferritin H chain from N-terminus
TTASTSQVRQNYHQDSEAAINRQINLELYASYVYLSMSYYFDRDDVALKNFAKYFLHQSHEEREHAEKLMKLQNQRGGRIFLQDIKGMHGKTQATSGTIQSGKPDCDDWESGLNAMECALHLEKNVNQSLLELHKLATDKNDPHLCDFIETHYLNEQVKAIKELGDHVTNLRKMGAPESGLAEYLFDKHTLGDSDNES